European Patent Application EP 4 234 029 A1, published August 30, 2023. Title: CHIMERIC ANTIGEN COMPRISING THE EXTRACELLULAR DOMAIN OF PD-L1. Applicant: CENTRO DE INGENIERIA GENETICA Y BIOTECNOLOGIA. Application CU 2020-0075. The sequence listing filed with the application follows.

SEQUENCE LISTING (24 sequences)

SEQ ID NO: 1 - protein, 290 aa, Artificial Sequence
  Description of Artificial Sequence: Quimeric antigen PKPD-L1
MVDKRMALVELKVPDIGGHENVDIIAVEVNVGDTIAVDDTLITLDLDHDDDDDKASDLLAFTVTVPKDLYVVEYGSNMTIECKFPVEKQLDLAALIVYWEMEDKNIIQFVHGEEDLKVQHSSYRQRARLLKDQLSLGNAALQITDVKLQDAGVYRCMISYGGADYKRITVKVNAPYNKINQRILVVDPVTSEHELTCQAEGYPKAEVIWTSSDHQVLSGKTTTTNSKREEKLFNVTSTLRINTTTNEIFYCTFRRLDPEENHTAELVIPELPLAHPPNERGSRAHHHHHH

SEQ ID NO: 2 - DNA, 31 bp, Homo sapiens
gatctgctagcctttaccgttaccgtcccga

SEQ ID NO: 3 - DNA, 60 bp, Homo sapiens
aatggtcatattgctgccatattctaccacatacaaatctttcgggacggtaacggtaaa

SEQ ID NO: 4 - DNA, 60 bp, Homo sapiens
aatatggcagcaatatgaccattgaatgcaaatttccggtggaaaaacagctggatctgg

SEQ ID NO: 5 - DNA, 60 bp, Homo sapiens
tattcttatcttccatttcccaatacacaattaacgccgccagatccagctgtttttcca

SEQ ID NO: 6 - DNA, 60 bp, Homo sapiens
tgtattgggaaatggaagataagaatatcattcagtttgtgcatggcgaagaagatctga

SEQ ID NO: 7 - DNA, 60 bp, Homo sapiens
agcagacgagcacgctgacgatagctgctatgctgcactttcagatcttcttcgccatgc

SEQ ID NO: 8 - DNA, 60 bp, Homo sapiens
agcgtgctcgtctgctgaaagatcaactgagcctgggcaatgcggcgctgcagattaccg

SEQ ID NO: 9 - DNA, 60 bp, Homo sapiens
ctaatcatgcaacgatacacgcccgcatcctgcagtttcacgtcggtaatctgcagcgcc

SEQ ID NO: 10 - DNA, 60 bp, Homo sapiens
gcgtgtatcgttgcatgattagctatggcggagcggactataaacgtattaccgtgaagg

SEQ ID NO: 11 - DNA, 60 bp, Homo sapiens
aatccgctggttaatcttattgtacggcgcattcaccttcacggtaatacgtttatagtc

SEQ ID NO: 12 - DNA, 60 bp, Homo sapiens
gtacaataagattaaccagcggattctggtggtggacccggtgaccagcgaacatgaact

SEQ ID NO: 13 - DNA, 60 bp, Homo sapiens
aatcacttccgctttcggatagccttccgcctggcaggtcagttcatgttcgctggtcac

SEQ ID NO: 14 - DNA, 60 bp, Homo sapiens
tatccgaaagcggaagtgatttggaccagcagcgatcatcaggtgctgtcaggcaagacc

SEQ ID NO: 15 - DNA, 60 bp, Homo sapiens
gacgttaaaaagcttctcctcgcgtttgctgttggtggtagtggtcttgcctgacagcac

SEQ ID NO: 16 - DNA, 59 bp, Homo sapiens
cgaggagaagctttttaacgtcaccagcaccctgcgtattaacactactaccaacgaaa

SEQ ID NO: 17 - DNA, 60 bp, Homo sapiens
ttccggatctaaacgacgaaaggtgcaatagaaaatttcgttggtagtagtgttaatacg

SEQ ID NO: 18 - DNA, 60 bp, Homo sapiens
tttcgtcgtttagatccggaagaaaatcataccgccgaactggtgattccggagctgccg

SEQ ID NO: 19 - DNA, 47 bp, Homo sapiens
ggatccacgttcattcggtggatgcgccagcggcagctccggaatca

SEQ ID NO: 20 - DNA, 31 bp, Artificial Sequence; identical to SEQ ID NO: 2
  Description of Artificial Sequence: Synthetic Oligonucleotide for cloning pM238

SEQ ID NO: 21 - DNA, 50 bp, Artificial Sequence
  Description of Artificial Sequence: Synthetic Oligonucleotide for cloning pM238
gggggatccacgttcattcggtggatgcgccagcggcagctccggaatca

SEQ ID NO: 22 - DNA, 870 bp, Artificial Sequence
  Description of Artificial Sequence: Nucleotide sequence of the coding region for the recombinant protein PKPD-L1
atggtagataaaagaatggctttagttgaattgaaagtgcccgacattggcggacacgaaaatgtagatattatcgcggttgaagtaaacgtgggcgacactattgctgtggacgataccctgattactttggatctagatcacgatgacgatgacgataaagcttcagatctgctagcctttaccgttaccgtcccgaaagatttgtatgtggtagaatatggcagcaatatgaccattgaatgcaaatttccggtggaaaaacagctggatctggcggcgttaattgtgtattgggaaatggaagataagaatatcattcagtttgtgcatggcgaagaagatctgaaagtgcagcatagcagctatcgtcagcgtgctcgtctgctgaaagatcaactgagcctgggcaatgcggcgctgcagattaccgacgtgaaactgcaggatgcgggcgtgtatcgttgcatgattagctatggcggagcggactataaacgtattaccgtgaaggtgaatgcgccgtacaataagattaaccagcggattctggtggtggacccggtgaccagcgaacatgaactgacctgccaggcggaaggctatccgaaagcggaagtgatttggaccagcagcgatcatcaggtgctgtcaggcaagaccactaccaccaacagcaaacgcgaggagaagctttttaacgtcaccagcaccctgcgtattaacactactaccaacgaaattttctattgcacctttcgtcgtttagatccggaagaaaatcataccgccgaactggtgattccggagctgccgctggcgcatccaccgaatgaacgtggatcccgggcacaccatcaccatcaccat

SEQ ID NO: 23 - protein, 19 aa, Homo sapiens
FMTYWHLLNAFTVTVPKDL

SEQ ID NO: 24 - protein, 23 aa, Homo sapiens
VILGAILLCLGVALTFIFRLRKG